European Patent Application EP 4 501 957 A1, published February 5, 2025. Title: ANTI-SERUM ALBUMIN NANOBODY AND DERIVATIVE THEREOF. Applicant: BIOTHEUS INC. Application WO PCT/CN2023/085559, filed March 31, 2023. The sequence listing filed with the application follows.

SEQUENCE LISTING (82 sequences)

SEQ ID NO: 1 - protein, 124 aa, synthetic construct
  source 1..124: note = VHH
QVQLQESGGGLVQPGGSLRLSCAAASGFTLDYYAIGWFRQAPGKEREGVSCISSSGGSTNSADSVKGRFTISRDNAKNTVYLQMNSLKPEDTAVYYCAAATLECRTVVVGYDYWGQGTQVTVSS

SEQ ID NO: 2 - protein, 115 aa, synthetic construct
  source 1..115: note = VHH
QVQLQESGGGLVQPGGSLRLSCKASGFTFSIYSMGWYRQVPGKEREAVATISSGGSPFYANSASGRFTISRDNAKSTVYLQMNNLKPEDTGVYSCSPITSIFKAQGQGTQVTVSS

SEQ ID NO: 3 - protein, 123 aa, synthetic construct
  source 1..123: note = VHH
QVQLQESGGGLVQAGGSLRLSCAASGFTLDYYAIGWFRQAPGKEREEVSCISSSGGSTNYADSVKGRFTISRDNAKNTVYLQMNSLKPEDTGVYYCAAALLECRVRSWPSDNWGQGTQVTVSS

SEQ ID NO: 4 - protein, 123 aa, synthetic construct
  source 1..123: note = VHH
EVQLLESGGGLVQPGGSLRLSCAASGFTLDYYAIGWFRQAPGKEREEVSCISSSGGSTNYADSVKGRFTISRDNSKNTVYLQMNSLKPEDTAVYYCAAALLECRVRSWPSDNWGQGTQVTVSS

SEQ ID NO: 5 - protein, 123 aa, synthetic construct
  source 1..123: note = VHH
EVQLLESGGGLVQPGGSLRLSCAASGFTLDYYAIGWFRQAPGKGLEEVSCISSSGGSTNYADSVKGRFTISRDNSKNTVYLQMNSLKPEDTAVYYCAAALLECRVRSWPSDNWGQGTQVTVSS

SEQ ID NO: 6 - protein, 123 aa, synthetic construct
  source 1..123: note = VHH
EVQLLESGGGLVQPGGSLRLSCAASGFTLDYYAIGWFRQAPGKEREEVSCISSSGGSTNYADSVKGRFTISRDNSKNTVYLQMNSLRAEDTAVYYCAAALLECRVRSWPSDNWGQGTQVTVSS

SEQ ID NO: 7 - protein, 115 aa, synthetic construct
  source 1..115: note = VHH
QVQLQESGGGLVQPGGSLRLSCAASGSIFTFYRMAWYRRAPGKERELVALITTDTSTNYADSVKGRFTISRDYAKNTVYLQMDSLKPEDTAAYYCNVRNVERDYWGQGTQVTVSS

SEQ ID NO: 8 - protein, 123 aa, synthetic construct
  source 1..123: note = VHH
QVQLQESGGGLVQPGGSLRLSCAASGFTLDYYAIGWFRQAPGKEREGVSCIASSGGSTNYADYVKGRFTISRDNAKNTVYLLMNKLKPEDTAVYYCAAAVLECRTVVREYDYWGQGTQVTVSS

SEQ ID NO: 9 - protein, 123 aa, synthetic construct
  source 1..123: note = VHH
QVQLQESGGGLVQPGGSLRLSCAASGFTLDYYAIGWFRQAPGKEREGVSCIASSGGSTNYADSVKGRFTISRDNAKNTVYLQMNKLKPEDTAVYYCAAAVLECRTVVRGYDYWGQGTQVTVSS

SEQ ID NO: 10 - protein, 123 aa, synthetic construct
  source 1..123: note = VHH
EVQLLESGGGLVQPGGSLRLSCAASGFTLDYYAIGWFRQAPGKEREGVSCIASSGGSTNYADSVKGRFTISRDNSKNTVYLQMNSLKPEDTAVYYCAAAVLECRTVVRGYDYWGQGTQVTVSS

SEQ ID NO: 11 - protein, 123 aa, synthetic construct
  source 1..123: note = VHH
EVQLLESGGGLVQPGGSLRLSCAASGETLDYYAIGWFRQAPGKEREGVSCIASSGGSTNYADSVKGRFTISRDNSKNTVYLQMNSLKPEDTAVYYCAAAVLECRTVVRGYDYWGQGTQVTVSS

SEQ ID NO: 12 - protein, 123 aa, synthetic construct
  source 1..123: note = VHH
EVQLLESGGGLVQPGGSLRLSCAASGFTLDYYAIGWFRQAPGKGLEGVSCIASSGGSTNYADSVKGRFTISRDNSKNTVYLQMNSLKPEDTAVYYCAAAVLECRTVVRGYDYWGQGTQVTVSS

SEQ ID NO: 13 - protein, 123 aa, synthetic construct
  source 1..123: note = VHH
EVQLLESGGGLVQPGGSLRLSCAASGFTLDYYAIGWFRQAPGKEREGVSCIASSGGSTNYADSVKGRFTISRDNSKNTVYLQMNSLRAEDTAVYYCAAAVLECRTVVRGYDYWGQGTQVTVSS

SEQ ID NO: 14 - protein, 123 aa, synthetic construct
  source 1..123: note = VHH
QVQLQESGGGLVQPGGSLRLSCVASRFTLDYYAIGWFRQAPGKEREGVSCIASSGGSTNYADSVKGRFTISRDNAKNTVYLQMNKLKPEDTAVYYCAAAVLECRTVVRGYDYWGQGTQVTVSS

SEQ ID NO: 15 - protein, 123 aa, synthetic construct
  source 1..123: note = VHH
QVQLQESGGGLVQPGGSLRLSCAASGFTLDYYAIGWFRQAPGKEREGVSCIASSGGSTNYADSVKGRFTISRDNAKNTVYLQMNSLKPEDTAVYYCAAATLECRTTLTGYAYWGQGTQVTVSS

SEQ ID NO: 16 - protein, 124 aa, synthetic construct
  source 1..124: note = VHH
QVQLQESGGGLVQPGGSLRLSCEAASGFTLDYYAIGWFRQAPGKEREGVSCISSSGGSTNSADSVKGRFTISRDNAKNTVYLQMNSLKPEDTAVYYCAAATLECRTVVVGYDYWGQGTQVTVSS

SEQ ID NO: 17 - protein, 122 aa, synthetic construct
  source 1..122: note = VHH
QVQLQESGGGLVQPGGSLRLSCTASGSTLDYYAIGWFRQAPGKEREGVSCISSSGGSTIYADSVKGRFTISRDNAKNTVYLQMNSLKPEDTAVYYCAAAVLECRAAEYVNSWGQGTQVTVSS

SEQ ID NO: 18 - protein, 123 aa, synthetic construct
  source 1..123: note = VHH
QVQLQESGGGLVQPGGSLRLSCAASRFTLDYYAIAWFRQAPGKDLEEVSCISSSGGATNYADSVKGRFTISRDNAKNTVYLQMNSLKPEETAVYYCAAATLECRGRSSSYDYWGQGTQVTVSS

SEQ ID NO: 19 - protein, 123 aa, synthetic construct
  source 1..123: note = VHH
QVQLQESGGGLVQPGGSLRLSCAASGFTLDYYAIAWFRQAPGKDLEGVSCIASSGGATNYADSVKGRFTISRDNAKNTVYLQMNKLKPEETAVYYCAAATFECRGRSSSYDYWGQGTQVTVSS

SEQ ID NO: 20 - protein, 123 aa, synthetic construct
  source 1..123: note = VHH
QVQLQESGGGLVQPGGSLRLSCAASRFTLDYYAIGWFRQAPGKEREGVSCIASSGGSTNYADSVKGRFTISRDNAKNTVYLQMNKLKPEDTAVYYCAAAVLECRTVVRGYDYWGQGTQVTVSS

SEQ ID NO: 21 - protein, 123 aa, synthetic construct
  source 1..123: note = VHH
QVQLQESGGGLVQPGGSLRLSCAASGFTLDYYAIGWFRQAPGKEREGVSCISSSGGSTNNADSVKGRFTISRDNAENTVYLQMNSLKPEDTAVYYCAAAVLECRTVVRGYDYWGQGTQVTVSS

SEQ ID NO: 22 - protein, 123 aa, synthetic construct
  source 1..123: note = VHH
QVQLQESGGGLVQPGGSLRLSCAASGFTLDYYAIGWFRQAPGKEREGVSCIASSGGSTNYADSVKGRFTISRDNAENTVYLQMNSLKPEDTAVYYCAAAVLECRTVVRGYDYWGQGTQVTVSS

SEQ ID NO: 23 - protein, 123 aa, synthetic construct
  source 1..123: note = VHH
QVQLQESGGGLVQPGGSLRLSCVASGFTLDYYAIGWFRQAPGKEREGVSCISSSGGSTNYADSVKGRFTISRDNAKNTVYLQMNSLKPEDTAVYYCAAAVLECRTVVRGYDYWGQGTQVTVSS

SEQ ID NO: 24 - protein, 115 aa, synthetic construct
  source 1..115: note = VHH
QVQLQESGGGLVQPGGSLRLSCVASGSIWGIYHMGWYRQAPGKQRELVASITVDGSTHYADTVKGRFTISKDNAANMVYLQMNALEPEDTAVYYCDIRNVGGDYWGQGTQVTVSS

SEQ ID NO: 25 - protein, 115 aa, synthetic construct
  source 1..115: note = VHH
QVQLVESGGGLVQPGGSLRLSCSASGSIWGIYHMGWYRQAPGKQRELVASITVDGSTHYADTVKGRFTISRDNSKNMVYLQMNSLEPEDTAVYYCDIRNVGGDYWGQGTQVTVSS

SEQ ID NO: 26 - protein, 115 aa, synthetic construct
  source 1..115: note = VHH
QVQLVESGGGLVQPGGSLRLSCSASGSIWGIYHMGWYRQAPGKGLELVASITVDGSTHYADTVKGRFTISRDNSKNMVYLQMNSLEPEDTAVYYCDIRNVGGDYWGQGTQVTVSS

SEQ ID NO: 27 - protein, 115 aa, synthetic construct
  source 1..115: note = VHH
QVQLVESGGGLVQPGGSLRLSCSASGSIWGIYHMGWYRQAPGKQRELVASITVDGSTHYADTVKGRFTISRDNSKNMVYLQMNSLRAEDTAVYYCDIRNVGGDYWGQGTQVTVSS

SEQ ID NO: 28 - protein, 123 aa, synthetic construct
  source 1..123: note = VHH
QVQLQESGGGLVQPGGSLRLSCAASGFTLDYYAIGWFRQAPGKEREGVSCISSSGGSTNYADSVKGRFTISKDNAKNTVYLQMNSLKPEDTAVYYCAAATLECRTVIRGYDYWGQGTQVTVSS

SEQ ID NO: 29 - protein, 123 aa, synthetic construct
  source 1..123: note = VHH
QVQLQESGGGLVQPGGSLRLSCTASGAQLEYYAIGWFRQAPGKEREGVSCISSSGGSTNNADSVKGRFTISRDNAKNTVYLQMNSLKPEDTAVYYCAAATLECRTVLTGYDYWGQGTQVTVSS

SEQ ID NO: 30 - protein, 9 aa, synthetic construct
  source 1..9: note = CDR1
SGFTLDYYA

SEQ ID NO: 31 - protein, 8 aa, synthetic construct
  source 1..8: note = CDR1
GFTFSIYS

SEQ ID NO: 32 - protein, 8 aa, synthetic construct
  source 1..8: note = CDR1
GFTLDYYA

SEQ ID NO: 33 - protein, 8 aa, synthetic construct
  source 1..8: note = CDR1
GSIFTFYR

SEQ ID NO: 34 - protein, 8 aa, synthetic construct
  source 1..8: note = CDR1
GETLDYYA

SEQ ID NO: 35 - protein, 8 aa, synthetic construct
  source 1..8: note = CDR1
RFTLDYYA

SEQ ID NO: 36 - protein, 8 aa, synthetic construct
  source 1..8: note = CDR1
GSTLDYYA

SEQ ID NO: 37 - protein, 8 aa, synthetic construct
  source 1..8: note = CDR1
GSIWGIYH

SEQ ID NO: 38 - protein, 8 aa, synthetic construct
  source 1..8: note = CDR1
GAQLEYYA

SEQ ID NO: 39 - protein, 8 aa, synthetic construct
  source 1..8: note = CDR2
ISSSGGST

SEQ ID NO: 40 - protein, 7 aa, synthetic construct
  source 1..7: note = CDR2
ISSGGSP

SEQ ID NO: 41 - protein, 8 aa, synthetic construct
  source 1..8: note = CDR2
ISSSGGST

SEQ ID NO: 42 - protein, 7 aa, synthetic construct
  source 1..7: note = CDR2
ITTDTST

SEQ ID NO: 43 - protein, 8 aa, synthetic construct
  source 1..8: note = CDR2
IASSGGST

SEQ ID NO: 44 - protein, 8 aa, synthetic construct
  source 1..8: note = CDR2
ISSSGGAT

SEQ ID NO: 45 - protein, 8 aa, synthetic construct
  source 1..8: note = CDR2
IASSGGAT

SEQ ID NO: 46 - protein, 7 aa, synthetic construct
  source 1..7: note = CDR2
ITVDGST

SEQ ID NO: 47 - protein, 16 aa, synthetic construct
  source 1..16: note = CDR3
AAATLECRTVVVGYDY

SEQ ID NO: 48 - protein, 9 aa, synthetic construct
  source 1..9: note = CDR3
SPITSIFKA

SEQ ID NO: 49 - protein, 16 aa, synthetic construct
  source 1..16: note = CDR3
AAALLECRVRSWPSDN

SEQ ID NO: 50 - protein, 9 aa, synthetic construct
  source 1..9: note = CDR3
NVRNVERDY

SEQ ID NO: 51 - protein, 16 aa, synthetic construct
  source 1..16: note = CDR3
AAAVLECRTVVREYDY

SEQ ID NO: 52 - protein, 16 aa, synthetic construct
  source 1..16: note = CDR3
AAAVLECRTVVRGYDY

SEQ ID NO: 53 - protein, 16 aa, synthetic construct
  source 1..16: note = CDR3
AAATLECRTTLTGYAY

SEQ ID NO: 54 - protein, 15 aa, synthetic construct
  source 1..15: note = CDR3
AAAVLECRAAEYVNS

SEQ ID NO: 55 - protein, 16 aa, synthetic construct
  source 1..16: note = CDR3
AAATLECRGRSSSYDY

SEQ ID NO: 56 - protein, 16 aa, synthetic construct
  source 1..16: note = CDR3
AAATFECRGRSSSYDY

SEQ ID NO: 57 - protein, 9 aa, synthetic construct
  source 1..9: note = CDR3
DIRNVGGDY

SEQ ID NO: 58 - protein, 16 aa, synthetic construct
  source 1..16: note = CDR3
AAATLECRTVIRGYDY

SEQ ID NO: 59 - protein, 16 aa, synthetic construct
  source 1..16: note = CDR3
AAATLECRTVLTGYDY

SEQ ID NO: 60 - DNA, 23 bp, synthetic construct
  source 1..23: mol_type = other DNA; note = upstream primer of the first round PCR
gtcctggctgctcttctacaagg

SEQ ID NO: 61 - DNA, 23 bp, synthetic construct
  source 1..23: mol_type = other DNA; note = downstream primer of the first round PCR
ggtacgtgctgttgaactgttcc

SEQ ID NO: 62 - DNA, 33 bp, synthetic construct
  source 1..33: mol_type = other DNA; note = upstream primer of the second round PCR
ctagtgcggccgcctggagacggtgacctgggt

SEQ ID NO: 63 - DNA, 38 bp, synthetic construct
  source 1..38: mol_type = other DNA; note = downstream primer of the second round PCR
cgcggatcccaggtgcagctgcaggagtctggrggagg

SEQ ID NO: 64 - DNA, 89 bp, synthetic construct
  source 1..89: mol_type = other DNA; note = upstream primer of the third round PCR
atttttactgctgttttattcgcagcatcctccgcattagctaaaagagaggctgaagcacaggtgcagctgcaggagtctggrggagg

SEQ ID NO: 65 - DNA, 81 bp, synthetic construct
  source 1..81: mol_type = other DNA; note = downstream primer of the third round PCR
agttgtcagttcctgtgccccccctcctcccgcgccacctccgcccgcacctccgccaccactggagacggtgacctgggt

SEQ ID NO: 66 - DNA, 60 bp, synthetic construct
  source 1..60: mol_type = other DNA; note = sequence of upstream homology arm
atttttactgctgttttattcgcagcatcctccgcattagctaaaagagaggctgaagca

SEQ ID NO: 67 - DNA, 60 bp, synthetic construct
  source 1..60: mol_type = other DNA; note = sequence of downstream homology arm
agttgtcagttcctgtgccccccctcctcccgcgccacctccgcccgcacctccgccacc

SEQ ID NO: 68 - protein, 226 aa, synthetic construct
  source 1..226: note = IgG1(LALA ) Fc
DKTHTCPPCPAPEAAGGPSVFLFPPKPKDTLMISRTPEVTCVVVDVSHEDPEVKFNWYVDGVEVHNAKTKPREEQYNSTYRVVSVLTVLHQDWLNGKEYKCKVSNKALPAPIEKTISKAKGQPREPQVYTLPPSRDELTKNQVSLTCLVKGFYPSDIAVEWESNGQPENNYKTTPPVLDSDGSFFLYSKLTVDKSRWQQGNVFSCSVMHEALHNHYTQKSLSLSPG

SEQ ID NO: 69 - protein, 501 aa, synthetic construct
  source 1..501: note = Bi-352
DIVMTQSPDSLAVSLGERATINCKSSQSLLNARTGKNYLAWYQQKPGQPPKLLIYWASTRESGVPDRFSGSGSGTDFTLTISSLQAEDVAVYYCKQSYSRRTFGGGTKVEIKRTVAAPSVFIFPPSDEQLKSGTASVVCLLNNFYPREAKVQWKVDNALQSGNSQESVTEQDSKDSTYSLSSTLTLSKADYEKHKVYACEVTHQGLSSPVTKSFNRGECGGGGSGGGGSGGGGSGGGGSGQVQLVESGGGLVQPGGSLRLSCSASGNSANIFSFASVAWYRQAPGKGLELVSVITSAGGTKYSDSVKGRFTISRDNSKNTLYLQMNSLRAEDTAVYYCNVDYLQDYWGQGTLVTVSSGGGGSGGGGSGGGGSGGGGSGEVQLLESGGGLVQPGGSLRLSCAASGFTLDYYAIGWFRQAPGKEREGVSCIASSGGSTNYADSVKGRFTISRDNSKNTVYLQMNSLKPEDTAVYYCAAAVLECRTVVRGYDYWGQGTQVTVSS

SEQ ID NO: 70 - protein, 501 aa, synthetic construct
  source 1..501: note = Bi-353
DIVMTQSPDSLAVSLGERATINCKSSQSLLNARTGKNYLAWYQQKPGQPPKLLIYWASTRESGVPDRFSGSGSGTDFTLTISSLQAEDVAVYYCKQSYSRRTFGGGTKVEIKRTVAAPSVFIFPPSDEQLKSGTASVVCLLNNFYPREAKVQWKVDNALQSGNSQESVTEQDSKDSTYSLSSTLTLSKADYEKHKVYACEVTHQGLSSPVTKSFNRGECGGGGSGGGGSGGGGSGGGGSGQVQLVESGGGLVQPGGSLRLSCSASGNSANIFSFASVAWYRQAPGKGLELVSVITSAGGTKYSDSVKGRFTISRDNSKNTLYLQMNSLRAEDTAVYYCNVDYLQDYWGQGTLVTVSSGGGGSGGGGSGGGGSGGGGSGEVQLLESGGGLVQPGGSLRLSCAASGFTLDYYAIGWFRQAPGKEREEVSCISSSGGSTNYADSVKGRFTISRDNSKNTVYLQMNSLKPEDTAVYYCAAALLECRVRSWPSDNWGQGTQVTVSS

SEQ ID NO: 71 - protein, 493 aa, synthetic construct
  source 1..493: note = Bi-354
DIVMTQSPDSLAVSLGERATINCKSSQSLLNARTGKNYLAWYQQKPGQPPKLLIYWASTRESGVPDRFSGSGSGTDFTLTISSLQAEDVAVYYCKQSYSRRTFGGGTKVEIKRTVAAPSVFIFPPSDEQLKSGTASVVCLLNNFYPREAKVQWKVDNALQSGNSQESVTEQDSKDSTYSLSSTLTLSKADYEKHKVYACEVTHQGLSSPVTKSFNRGECGGGGSGGGGSGGGGSGGGGSGQVQLVESGGGLVQPGGSLRLSCSASGNSANIFSFASVAWYRQAPGKGLELVSVITSAGGTKYSDSVKGRFTISRDNSKNTLYLQMNSLRAEDTAVYYCNVDYLQDYWGQGTLVTVSSGGGGSGGGGSGGGGSGGGGSGQVQLVESGGGLVQPGGSLRLSCSASGSIWGIYHMGWYRQAPGKQRELVASITVDGSTHYADTVKGRFTISRDNSKNTLYLQMNSLEPEDTAVYYCDIRNVGGDYWGQGTQVTVSS

SEQ ID NO: 72 - skipped

SEQ ID NO: 73 - protein, 8 aa, synthetic construct
  source 1..8: note = Formula II
  VARIANT 2: note = X is selected from (i) amino acid residues A, S; and (ii) amino acid residues that are conservative substitutions relative to (i).
  VARIANT 7: note = X is selected from (i) amino acid residues A, S; and (ii) amino acid residues that are conservative substitutions relative to (i).
  VARIANT 8: note = X is selected from (i) amino acid residue T; and (ii) amino acid residues that are conservative substitutions relative to (i).
IXSSGGXX

SEQ ID NO: 74 - protein, 16 aa, synthetic construct
  source 1..16: note = Forluma III
  VARIANT 4: note = X is selected from (i) amino acid residues T, V; and (ii) amino acid residues that are conservative substitutions relative to (i).
  VARIANT 10: note = X is selected from (i) amino acid residues T, V; and (ii) amino acid residues that are conservative substitutions relative to (i).
  VARIANT 11: note = X is selected from (i) amino acid residues V, I, L; and (ii) amino acid residues that are conservative substitutions relative to (i).
  VARIANT 12: note = X is selected from (i) amino acid residues R, V, T; and (ii) amino acid residues that are conservative substitutions relative to (i).
  VARIANT 13: note = X is selected from (i) amino acid residues G, E; and (ii) amino acid residues that are conservative substitutions relative to (i).
  VARIANT 15: note = X is selected from (i) amino acid residues D, A; and (ii) amino acid residues that are conservative substitutions relative to (i).
AAAXLECRTXXXXYXY

SEQ ID NO: 75 - protein, 16 aa, synthetic construct
  source 1..16: note = Formula IV
  VARIANT 5: note = X is selected from (i) amino acid residues L, F; and (ii) amino acid residues that are conservative substitutions relative to (i).
AAATXECRGRSSSYDY

SEQ ID NO: 76 - protein, 365 aa, synthetic construct
  source 1..365: note = Bi-340
QVQLVQSGAEVKKPGASVKVSCKASGFNIKDYYMHWVRQAPGQRLEWMGWIDLEEGNTIYDAKFQGRVTITRDTSASTAYMELSSLRSEDTAVYYCARDAYGRYFYDVWGQGTLVTVSSASTKGPSVFPLAPSSKSTSGGTAALGCLVKDYFPEPVTVSWNSGALTSGVHTFPAVLQSSGLYSLSSVVTVPSSSLGTQTYICNVNHKPSNTKVDKKVEPKSCDKTHTGGGGSGGGGSGGGGSGGGGSGQVQLVESGGGLVQPGGSLRLSCSASGNSANIFSFASVAWYRQAPGKGLELVSVITSAGGTKYSDSVKGRFTISRDNSKNTLYLQMNSLRAEDTAVYYCNVDYLQDYWGQGTLVTVSS

SEQ ID NO: 77 - protein, 493 aa, synthetic construct
  source 1..493: note = Bi-356
DIVMTQSPDSLAVSLGERATINCKSSQSLLNARTGKNYLAWYQQKPGQPPKLLIYWASTRESGVPDRFSGSGSGTDFTLTISSLQAEDVAVYYCKQSYSRRTFGGGTKVEIKRTVAAPSVFIFPPSDEQLKSGTASVVCLLNNFYPREAKVQWKVDNALQSGNSQESVTEQDSKDSTYSLSSTLTLSKADYEKHKVYACEVTHQGLSSPVTKSFNRGECGGGGSGGGGSGGGGSGGGGSGQVQLVESGGGLVQPGGSLRLSCSASGNSANIFSFASVAWYRQAPGKGLELVSVITSAGGTKYSDSVKGRFTISRDNSKNTLYLQMNSLRAEDTAVYYCNVDYLQDYWGQGTLVTVSSGGGGSGGGGSGGGGSGGGGSGEVQLQESGGGLVQPGGSLRLSCAASGFTFSSYWMYWLRQAPGKGLEWVSSINSDSSSTYYRDSVKGRFTISRDNAKNTLYLQMNSLKSEDTAVYYCAKDPGGYAKGQGTQVTVSS

SEQ ID NO: 78 - protein, 115 aa, synthetic construct
  source 1..115: note = VHH
QVQLVESGGGLVQPGGSLRLSCSASGSIWGIYHMGWYRQAPGKQRELVASITVDGSTHYADTVKGRFTISRDNSKNTLYLQMNSLEPEDTAVYYCDIRNVGGDYWGQGTQVTVSS

SEQ ID NO: 79 - protein, 219 aa, synthetic construct
  source 1..219: note = light chain of anti-secondary antigen Fab
DIVMTQSPDSLAVSLGERATINCKSSQSLLNARTGKNYLAWYQQKPGQPPKLLIYWASTRESGVPDRFSGSGSGTDFTLTISSLQAEDVAVYYCKQSYSRRTFGGGTKVEIKRTVAAPSVFIFPPSDEQLKSGTASVVCLLNNFYPREAKVQWKVDNALQSGNSQESVTEQDSKDSTYSLSSTLTLSKADYEKHKVYACEVTHQGLSSPVTKSFNRGEC

SEQ ID NO: 80 - protein, 227 aa, synthetic construct
  source 1..227: note = heavy chain of anti-secondary antigen Fab
QVQLVQSGAEVKKPGASVKVSCKASGFNIKDYYMHWVRQAPGQRLEWMGWIDLEEGNTIYDAKFQGRVTITRDTSASTAYMELSSLRSEDTAVYYCARDAYGRYFYDVWGQGTLVTVSSASTKGPSVFPLAPSSKSTSGGTAALGCLVKDYFPEPVTVSWNSGALTSGVHTFPAVLQSSGLYSLSSVVTVPSSSLGTQTYICNVNHKPSNTKVDKKVEPKSCDKTHT

SEQ ID NO: 81 - protein, 117 aa, synthetic construct
  source 1..117: note = VHH of anti-third antigen nanobody
QVQLVESGGGLVQPGGSLRLSCSASGNSANIFSFASVAWYRQAPGKGLELVSVITSAGGTKYSDSVKGRFTISRDNSKNTLYLQMNSLRAEDTAVYYCNVDYLQDYWGQGTLVTVSS

SEQ ID NO: 82 - protein, 115 aa, synthetic construct
  source 1..115: note = VHH of non-HSA-associated nanobody
EVQLQESGGGLVQPGGSLRLSCAASGFTFSSYWMYWLRQAPGKGLEWVSSINSDSSSTYYRDSVKGRFTISRDNAKNTLYLQMNSLKSEDTAVYYCAKDPGGYAKGQGTQVTVSS